European Patent Specification EP 4 023 771 B1, published March 4, 2026. Title: Method for Identifying Whether a Diploid Potato Is Self-Compatible. Applicant: YUNNAN NORMAL UNIVERSITY. The sequence listing filed with the application follows.

SEQUENCE LISTING (12 sequences)

SEQ ID NO: 1 - DNA, 4289 bp, Unknown
  nucleotide sequence of the StSCI gene
atctcgagttaatttcacatttgatcactgaacttttcccactataagtgactacatgttatccactcttaacactacgtgcctcgacaattttaggtgaaaagtctaaattacttaactttttctatcttgcagatttccattgaaatcccatatgtctttatgcaatctgttttctgtggtgcaattatgtatgctatgatcggatttgaatggacggtagcaaagttcttttggtacttgttcttcctgtttttcaccctcttgtacttcactttctacggtatgatgaccgttgctgttaccccaaatgtaagtgttgctcaaattgtcggctccttcttctacggagtatggaatcttttctcaggattcatcattccacgaactgtaagttcttgaaacacttccattttattgttacatcaaaactgacttagagctcggaaatgacatgttctctgtatttttttccattttcatttttaaaaaacagcgtattcccatatggtggagatggtactactggtgttgtcctgttgcctggaccttgtatggtttggttgcatcacaatttggagatcttcagaacaaacttactgatgaggaaacagtggaacaatttttgagacgttacttcggcttcaagcatgattttcttccaatagttgcagtcgcgattgttgggtacactgttctttttggcttcacatttgctttcgctattaaggcattcaacttccaaacgagataaaaagacattacctgctgaagatgtagtaaagacaacgtgtgaaacgttctctccactgctcgtgaaatggggaagacgcggttagtataaggaatttttctcgagctcaagtacgagcaagagattgattttgaaagtactgtatatagattaccacttgaacaagggtatgttctgttattattattattttttatgaatttcaagttcatttttctgtgtaagagatagtaatttgttaatgttgaagtactattctgttactatctggtgtttcttgtacttttgttgtgtctttttctgaactgctttggattatttttctcgagtcgaggatctatcggaagaagactttctacctctgaggtaagagtaaagtttgcttacactctacccttcccatactccactttgtgggggagacacatggtatgttgttcttatagttacaactataagaaattaatgaaatgatgaatgtaagaatttgtgaatattgcttttcgggaactgccacaactgtggtgcgagaatgagacttctctagtgttaactaaacaacaagtctttggtttgaattcggagaatggagaaattcttggtcgggaacgctccttgataaatggaccttagatgatgctaatcttaaattagtcgggccagtaaatttcgaatcttccaagacatttcatgttttaattcactaaaaaggaaagacaaaaaatttcaaactcaaaacatttcatgtttagtattattggaatatcttcctccacatgagttgtttgtttggtgtatctaagcaatatcaattctttaattttatttttttttggaaataaaatgtacatatgtgagaactagataaaaataatgaaaaataaacaaaaatgatttttttaaaaataaaataaaattaaatattttcacttccattaggccaaaagggtatatctaggctatttgtgtaatagtataggtatgtatgagccatttttataacgaggtatgtatcagctctaaattatatgaccttttcacttattatattcatactggagaagtaaaaatgaacaaaacaatatttaaccgcagtgccggctcaatgcttataaaaattaggcatatgccttaggcccccaattttaggggggcctcaaatttttaccaacaataaattatgtgttaattttttttatagaaaaaattaattatttaagataaatgtacttttcatatatatattattttattctccttaacctcaatcaaatagaagaaatcaagaaaaacgttgttttgtcttcttacactctcttcacttactctcgcgttgtaattttctataccccttttatactctatgtaagttagagctctatcaaaaatatgaatcaatagtaaaactaatgtgttggataaagcgaattacaagcctgtttagattgacttatgttatgtgcttttaaataaaaaaagaagtttataagcagttttgtcaacttattacttatagaataatgttaacaatttatttaataattgcctcagctaaaagattttaggcctttaatttaaattttgttttaggcctccaaatacgttgagccgcccctgcttaaccgtcgagacatatgaagtgtaacaacttttcaacaaacttttctcagtttgctttatataaagaaaaaaaattcacaaaacttcaaattcaattttccaataatggactatttcctattgctaccagaagattgtgtttgtgatattctctcctttacttccccgaaagacgtcgtgatttcatccgcgatctctcggggattcaactctgctgctgaatccgacgttatttgggtaaagtttttaccagatgattatgaagatatcaactcgagatatgtctccccgcggatttatccgtctaaaaaggagctttactttagtctatgtgacttccctgttctaatggatggaggcaaattggtaagtagctctaaattgggaagtagcaagcttttcttttggctcattagttgaatatatgtataattgttttgaagcttatgggttcgggattttttgtgtgttttttgagttgtttggttcgaaattaataatttggtacaaattagaggagttttctttttaaagataaaatacagagtttgaactaaaactattgggttcctagaatttataggggtgttctagctttgcctctaactgttggtgttgtataacggtaaaggtcatgaacctttgacctgaggtctagagtttgagttttaatcagagttgaaatcttaggaattgagtcgtgtttaataggaagcactaaaatctactagtgtgcttacggctgcgcaaatcttaattaatcagccaatgaatttttcttattttattttgtttttgttacaaactgggaatccaactctctatagtaaaacggaagttcagatagtcaactaaatgaacttctaagattttctggccaatgggttacaaacaccattaaaaatgcaaaattaaatagattataataataattgtgtgaattttattttatttttgaatggactatatataagctagtagtgtgaatctaagattttattttatttttgaaaacagagtttttcacttgataagaaaacaggcaagaaatgttttatgatatcagctagagaacttgctattacatggggagttgatacaccatggtattgggaatggatttctcatcctgactccaggttcgtcgaaaaattatactacatataaaaagttattctttttttttatgtatgtactacgtataaaaaattatacttcattgccttttaacgaatttctacatatgttattttttgaatcccttggttgaaattctacctctgccactattggtgagaattttttttttacacaatcaagccacctaaaagatatatatagatgagcctcactaaaatgtgtaatgaaatatgttacctattacaataggtaaagatgatttgatggtgcaaaaattacttatattggcgatgttatatataacttaaactcactaaatacgtgtatctaagacaatatagacattttattttgcagattttcggaagtggctcatctcaagggtgtaagttggctagacatacgaggcacgattggaacacaaatattgtcgaaaagaaccaaatatgttgtttatttggtgttcaaattgtcaaagaatcatgatggactagaaattgctaatgcatttgttaggtttgtgaatcgtgtgagcgacaaagaggccgaggaacgagctagtgtcgtgagtctagtcggaaaaagggttaggagacgcaaacgtaatgtgaaatgtccacgaaaaagagtcgatggatggatggaaatagaattgggaaattttatcaatgatacaggagatgatggagatgttgaagcgcgattgatggagattacgcagcttcatggaaaaggtggccttattgttcaaggaattgaatttagaccagaataa

SEQ ID NO: 2 - DNA, 538 bp, Unknown
  nucleotide sequence of the inserted sequence
caggggcggctcaacgtatttggaggcctaaaacaaaatttaaattaaaggcctaaaatcttttagctgaggcaattattaaataaattgttaacattattctataagtaataagttgacaaaactgcttataaacttctttttttatttaaaagcacataacataagtcaatctaaacaggcttgtaattcgctttatccaacacattagttttactattgattcatatttttgatagagctctaacttacatagagtataaaaggggtatagaaaattacaacgcgagagtaagtgaagagagtgtaagaagacaaaacaacgtttttcttgatttcttctatttgattgaggttaaggagaataaaataatatatatatgaaaagtacatttatcttaaataattaattttttctataaaaaaaattaacacataatttattgttggtaaaaatttgaggcccccctaaaattgggggcctaaggcatatgcctaatttttataagcattgagccggcactgcggttaaatattg

SEQ ID NO: 3 - DNA, 101 bp, Artificial Sequence
  KASP primer sequence
ttatgatcttgataaactatatattatcaatatgaatgttgtaattgatatattattttgaactttgtccaatctatattagttatttaagtcatcatatt

SEQ ID NO: 4 - DNA, 101 bp, Artificial Sequence
  KASP primer sequence
ttatgatcttgataaactatatattatcaatatgaatgttgtaattgatacattattttgaactttgtccaatctatattagttatttaagtcatcatatt

SEQ ID NO: 5 - DNA, 20 bp, Artificial Sequence
  primer sequence
ggtgtatcgagtcggaataa

SEQ ID NO: 6 - DNA, 20 bp, Artificial Sequence
  primer sequence
gattcgggaaattgtactca

SEQ ID NO: 7 - DNA, 22 bp, Artificial Sequence
  the first forward primer 1F
cgtcggattcagcagcagagtt

SEQ ID NO: 8 - DNA, 27 bp, Artificial Sequence
  the first reverse primer 1R
tccacatgagttgtttgtttggtgtat

SEQ ID NO: 9 - DNA, 22 bp, Artificial Sequence
  the second forward primer 2F
cgtcggattcagcagcagagtt

SEQ ID NO: 10 - DNA, 29 bp, Artificial Sequence
  the second reverse primer 2R
aagcgaattacaagcctgtttagattgac

SEQ ID NO: 11 - DNA, 29 bp, Artificial Sequence
  primer sequence
atcagctagagaacttgctatttcatggg

SEQ ID NO: 12 - DNA, 26 bp, Artificial Sequence
  primer sequence
cgtgcctcgtatgtctagccaactta